European Patent Application EP 4 520 818 A1, published March 12, 2025. Title: BACULOVIRUS VECTOR AND USE THEREOF IN PREPARATION OF RECOMBINANT ADENO-ASSOCIATED VIRUS (rAAV) IN INSECT CELL. Applicant: GENEVOYAGER (WUHAN) CO., LTD. The sequence listing filed with the application follows.

SEQUENCE LISTING (7 sequences)

SEQ ID NO: 1 - DNA, 1590 bp, Artificial Sequence
  Expression cassette for homologous recombinant
tgctcctgacgccgctcctgacggcgatggctgcgactgcttgaagacggctggctgcgactgcttgaagacggctgggcttcgggagatgttgtaaagttgatgcggcgacggctgagagacagcctgtggcggcggctgctgctgggagtggcggcgttgatttggcgactcatggctgggctggtaggatactgttcactaggctgtgaggcttgaactgtgcttacgagtagaacggcagctgtatttatactgtttatcagtactgcacgactgataagacaatagtggtgggggaacttgccaggcaaaaatgagaagttcctatactttctagagaataggaacttcatttaaatggcgcgccttacgccccgccctgccactcatcgcagtactgttgtattcattaagcatctgccgacatggaagccatcacaaacggcatgatgaacctgaatcgccagcggcatcagcaccttgtcgccttgcgtataatatttgcccatggtgaaaacgggggcgaagaagttgtccatattggccacgtttaaatcaaaactggtgaaactcacccagggattggctgagacgaaaaacatattctcaataaaccctttagggaaataggccaggttttcaccgtaacacgccacatcttgcgaatatatgtgtagaaactgccggaaatcgtcgtggtattcactccagagcgatgaaaacgtttcagtttgctcatggaaaacggtgtaacaagggtgaacactatcccatatcaccagctcaccgtctttcattgccatacgtaattccggatgagcattcatcaggcgggcaagaatgtgaataaaggccggataaaacttgtgcttatttttctttacggtctttaaaaaggccgtaatatccagctgaacggtctggttataggtacattgagcaactgactgaaatgcctcaaaatgttctttacgatgccattgggatatatcaacggtggtatatccagtgatttttttctccattttagcttccttagctcctgaaaatctcgacaactcaaaaaatacgcccggtagtgatcttatttcattatggtgaaagttggaacctcttacgtgccgatcaacgtctcattttcgccaaaagttggcccagggcttcccggtatcaacagggacaccaggatttatttattctgcgaagtgatcttccgtcacaggtaggcgcgccgaagttcctatactttctagagaataggaacttctcattttaaatttatcatatcacaggctgcagtttctgttatctgtcccccactcaggcgtgcagctataaaagcaggcactcaccaactcgtaagcacagttcgttgtgaagtgaacacggagagcctgccaataagcaaaatgccaagggacaccaacaatcgccaccggtctacgccatatgaacgtcctacgcttgaagatctccgcagacagttgcaagacaatttggacagcataaaccgccgagacagaatgcaagaagaacaagaagaaaacctgcgctatcaagtgcgtagaaggcagcgtcaaaaccagc

SEQ ID NO: 2 - DNA, 1277 bp, Artificial Sequence
  Expression cassette homologous recombinant
cacccgacgtaataggctacgtgtcggatattatgcaaaacacttatattgtaacgtggttcaacaccgtcgacctttccacctatcacgaaagcgtgcatgatgaccggattgaaatttttgatttcttaaatcaaaaatttcaacctgttgatcgaatcgtacacgatcgcgttagagcaaatgatgaaaatcccaacgaagttcctatactttctagagaataggaacttcatttaaatggcgcgccttacgccccgccctgccactcatcgcagtactgttgtattcattaagcatctgccgacatggaagccatcacaaacggcatgatgaacctgaatcgccagcggcatcagcaccttgtcgccttgcgtataatatttgcccatggtgaaaacgggggcgaagaagttgtccatattggccacgtttaaatcaaaactggtgaaactcacccagggattggctgagacgaaaaacatattctcaataaaccctttagggaaataggccaggttttcaccgtaacacgccacatcttgcgaatatatgtgtagaaactgccggaaatcgtcgtggtattcactccagagcgatgaaaacgtttcagtttgctcatggaaaacggtgtaacaagggtgaacactatcccatatcaccagctcaccgtctttcattgccatacgtaattccggatgagcattcatcaggcgggcaagaatgtgaataaaggccggataaaacttgtgcttatttttctttacggtctttaaaaaggccgtaatatccagctgaacggtctggttataggtacattgagcaactgactgaaatgcctcaaaatgttctttacgatgccattgggatatatcaacggtggtatatccagtgatttttttctccattttagcttccttagctcctgaaaatctcgacaactcaaaaaatacgcccggtagtgatcttatttcattatggtgaaagttggaacctcttacgtgccgatcaacgtctcattttcgccaaaagttggcccagggcttcccggtatcaacagggacaccaggatttatttattctgcgaagtgatcttccgtcacaggtaggcgcgccgaagttcctatactttctagagaataggaacttcgcacgtcaaaaacggccaatacatggcgtgtcccgaagaattgtacgataacaacgaatttaaatgtaacatagaatcggataaattatactatttggataatttacaagaagattccattgtataa

SEQ ID NO: 3 - DNA, 2211 bp, Artificial Sequence
  Cap gene
ctggctgccgacggttatctacccgattggctcgaggacaaccttagtgaaggaattcgcgagtggtgggctttgaaacctggagcccctcaacccaaggcaaatcaacaacatcaagacaacgctcgaggtcttgtgcttccgggttacaaataccttggacccggcaacggactcgacaagggggagccggtcaacgcagcagacgcggcggccctcgagcacgacaaggcctacgaccagcagctcaaggccggagacaacccgtacctcaagtacaaccacgccgacgccgagttccaggagcggctcaaagaagatacgtcttttgggggcaacctcgggcgagcagtcttccaggccaaaaagaggcttcttgaacctcttggtctggttgaggaagcggctaagacggctcctggaaagaagaggcctgtagagcagtctcctcaggaaccggactcctccgcgggtattggcaaatcgggtgcacagcccgctaaaaagagactcaatttcggtcagactggcgacacagagtcagtcccagaccctcaaccaatcggagaacctcccgcagccccctcaggtgtgggatctcttacaatggcttcaggtggtggcgcaccagtggcagacaataacgaaggtgccgatggagtgggtagttcctcgggaaattggcattgcgattcccaatggctgggggacagagtcatcaccaccagcacccgaacctgggccctgcccacctacaacaatcacctctacaagcaaatctccaacagcacatctggaggatcttcaaatgacaacgcctacttcggctacagcaccccctgggggtattttgacttcaacagattccactgccacttctcaccacgtgactggcagcgactcatcaacaacaactggggattccggcctaagcgactcaacttcaagctcttcaacattcaggtcaaagaggttacggacaacaatggagtcaagaccatcgccaataaccttaccagcacggtccaggtcttcacggactcagactatcagctcccgtacgtgctcgggtcggctcacgagggctgcctcccgccgttcccagcggacgttttcatgattcctcagtacgggtatctgacgcttaatgatggaagccaggccgtgggtcgttcgtccttttactgcctggaatatttcccgtcgcaaatgctaagaacgggtaacaacttccagttcagctacgagtttgagaacgtacctttccatagcagctacgctcacagccaaagcctggaccgactaatgaatccactcatcgaccaatacttgtactatctctcaaagactattaacggttctggacagaatcaacaaacgctaaaattcagtgtggccggacccagcaacatggctgtccagggaagaaactacatacctggacccagctaccgacaacaacgtgtctcaaccactgtgactcaaaacaacaacagcgaatttgcttggcctggagcttcttcttgggctctcaatggacgtaatagcttgatgaatcctggacctgctatggccagccacaaagaaggagaggaccgtttctttcctttgtctggatctttaatttttggcaaacaaggaactggaagagacaacgtggatgcggacaaagtcatgataaccaacgaagaagaaattaaaactactaacccggtagcaacggagtcctatggacaagtggccacaaaccaccagagtgcccaagcacaggcgcagaccggctgggttcaaaaccaaggaatacttccgggtatggtttggcaggacagagatgtgtacctgcaaggacccatttgggccaaaattcctcacacggacggcaactttcacccttctccgctgatgggagggtttggaatgaagcacccgcctcctcagatcctcatcaaaaacacacctgtacctgcggatcctccaacggccttcaacaaggacaagctgaactctttcatcacccagtattctactggccaagtcagcgtggagatcgagtgggagctgcagaaggaaaacagcaagcgctggaacccggagatccagtacacttccaactattacaagtctaataatgttgaatttgctgttaatactgaaggtgtatatagtgaaccccgccccattggcaccagatacctgactcgtaatctgtaa

SEQ ID NO: 4 - DNA, 1866 bp, Artificial Sequence
  Rep gene
ctggcggggttttacgagattgtgattaaggtccccagcgaccttgacgggcatctgcccggcatttctgacagctttgtgaactgggtggccgagaaggagtgggagttgccgccagattctgacttggatctgaatctgattgagcaggcacccctgaccgtggccgagaagctgcagcgcgactttctgacggagtggcgccgtgtgagtaaggccccggaggcccttttctttgtgcaatttgagaagggagagagctacttccacttacacgtgctcgtggaaaccaccggggtgaaatccttagttttgggacgtttcctgagtcagattcgcgaaaaactgattcagagaatttaccgcgggatcgagccgactttgccaaactggttcgcggtcacaaagaccagaaacggcgccggaggcgggaacaaggtggtggacgagtgctacatccccaattacttgctccccaaaacccagcctgagctccagtgggcgtggactaatttagaacagtatttaagcgcctgtttgaatctcacggagcgtaaacggttggtggcgcagcatctgacgcacgtgtcgcagacgcaggagcagaacaaagagaatcagaatcccaattctgacgcgccggtgatcagatcaaaaacttcagccaggtacatggagctggtcgggtggctcgtggacaaggggattacctcggagaagcagtggatccaggaggaccaggcctcatacatctccttcaatgcggcctccaactcgcggtcccaaatcaaggctgccttggacaatgcgggaaagattatgagcctgactaaaaccgcccccgactacctggtgggccagcagcccgtggaggacatttccagcaatcggatttataaaattttggaactaaacgggtacgatccccaatatgcggcttccgtctttctgggatgggccacgaaaaagttcggcaagaggaacaccatctggctgtttgggcctgcaactaccgggaagaccaacatcgcggaggccatagcccacactgtgcccttctacgggtgcgtaaactggaccaatgagaactttcccttcaacgactgtgtcgacaagatggtgatctggtgggaggaggggaagatgaccgccaaggtcgtggagtcggccaaagccattctcggaggaagcaaggtgcgcgtggaccagaaatgcaagtcctcggcccagatagacccgactcccgtgatcgtcacctccaacaccaacatgtgcgccgtgattgacgggaactcaacgaccttcgaacaccagcagccgttgcaagaccggatgttcaaatttgaactcacccgccgtctggatcatgactttgggaaggtcaccaagcaggaagtcaaagactttttccggtgggcaaaggatcacgtggttgaggtggagcatgaattctacgtcaaaaagggtggagccaagaaaagacccgcccccagtgacgcagatataagtgagcccaaacgggtgcgcgagtcagttgcgcagccatcgacgtcagacgcggaagcttcgatcaactacgcagacaggtaccaaaacaaatgttctcgtcacgtgggcatgaatctgatgctgtttccctgcagacaatgcgagagaatgaatcagaattcaaatatctgcttcactcacggacagaaagactgtttagagtgctttcccgtgtcagaatctcaacccgtttctgtcgtcaaaaaggcgtatcagaaactgtgctacattcatcatatcatgggaaaggtgccagacgcttgcactgcctgcgatctggtcaatgtggatttggatgactgcatctttgaacaataa

SEQ ID NO: 5 - DNA, 156 bp, Artificial Sequence
  CNE
acttttttgtaatgcaaaaaagttgatagtgtagtagtatattgggagcgtatcgtacagtgtagactattctaataaaatagtctacgatttgtagagattgtactgtatatggagtgtcaggcaaaagtgaacttttttgcattgcaaaaaaat

SEQ ID NO: 6 - DNA, 2407 bp, Artificial Sequence
  ITR-GOI
cctgcaggcagctgcgcgctcgctcgctcactgaggccgcccgggcaaagcccgggcgtcgggcgacctttggtcgcccggcctcagtgagcgagcgagcgcgcagagagggagtggccaactccatcactaggggttcctgcggccgcacgcgccgcccgtcagtgggcagagcgcacatcgcccacagtccccgagaagttggggggaggggtcggcaattgaaccggtgcctagagaaggtggcgcggggtaaactgggaaagtgatgtcgtgtactggctccgcctttttcccgagggtgggggagaaccgtatataagtgcagtagtcgccgtgaacgttctttttcgcaacgggtttgccgccagaacacgcgtaagggatccgccaccatggtgagcaagggcgaggaggataacatggccatcatcaaggagttcatgcgcttcaaggtgcacatggagggctccgtgaacggccacgagttcgagatcgagggcgagggcgagggccgcccctacgagggcacccagaccgccaagctgaaggtgaccaagggtggccccctgcccttcgcctgggacatcctgtcccctcagttcatgtacggctccaaggcctacgtgaagcaccccgccgacatccccgactacttgaagctgtccttccccgagggcttcaagtgggagcgcgtgatgaacttcgaggacggcggcgtggtgaccgtgacccaggactcctccctgcaggacggcgagttcatctacaaggtgaagctgcgcggcaccaacttcccctccgacggccccgtaatgcagaagaagaccatgggctgggaggcctcctccgagcggatgtaccccgaggacggcgccctgaagggcgagatcaagcagaggctgaagctgaaggacggcggccactacgacgctgaggtcaagaccacctacaaggccaagaagcccgtgcagctgcccggcgcctacaacgtcaacatcaagttggacatcacctcccacaacgaggactacaccatcgtggaacagtacgaacgcgccgagggccgccactccaccggcggcatggacgagctgtacaagtaagaattcgatatcaagcttatcgataatcaacctctggattacaaaatttgtgaaagattgactggtattcttaactatgttgctccttttacgctatgtggatacgctgctttaatgcctttgtatcatgctattgcttcccgtatggctttcattttctcctccttgtataaatcctggttgctgtctctttatgaggagttgtggcccgttgtcaggcaacgtggcgtggtgtgcactgtgtttgctgacgcaacccccactggttggggcattgccaccacctgtcagctcctttccgggactttcgctttccccctccctattgccacggcggaactcatcgccgcctgccttgcccgctgctggacaggggctcggctgttgggcactgacaattccgtggtgttgtcggggaaatcatcgtcctttccttggctgctcgcctgtgttgccacctggattctgcgcgggacgtccttctgctacgtcccttcggccctcaatccagcggaccttccttcccgcggcctgctgccggctctgcggcctcttccgcgtcttcgccttcgccctcagacgagtcggatctccctttgggccgcctccccgcatcgataccgagcgctgctcgagagatctacgggtggcatccctgtgacccctccccagtgcctctcctggccctggaagttgccactccagtgcccaccagccttgtcctaataaaattaagttgcatcattttgtctgactaggtgtccttctataatattatggggtggaggggggtggtatggagcaaggggcaagttgggaagacaacctgtagggcctgcggggtctattgggaaccaagctggagtgcagtggcacaatcttggctcactgcaatctccgcctcctgggttcaagcgattctcctgcctcagcctcccgagttgttgggattccaggcatgcatgaccaggctcagctaatttttgtttttttggtagagacggggtttcaccatattggccaggctggtctccaactcctaatctcaggtgatctacccaccttggcctcccaaattgctgggattacaggcgtgaaccactgctcccttccctgtccttctgattttgtaggtaaccacgtgcggaccgagcggccgcaggaacccctagtgatggagttggccactccctctctgcgcgctcgctcgctcactgaggccgggcgaccaaaggtcgcccgacgcccgggctttgcccgggcggcctcagtgagcgagcgagcgcgcagctgcctgcagg

SEQ ID NO: 7 - DNA, 200 bp, Artificial Sequence
  NAE
cattttcagcgacgtatattgacaaatatactacagtcggacgtttgtgccgacctatatactacactttaccaaaaatatactacactaaactctaaatatactacaactccacttcaatataaccacactctcgtaaaacggcccaaaaatatcgaaatatatggggcaaatacacgtttaaaaaacgctacgattcc